European Patent Application EP 4 722 366 A1, published April 8, 2026. Title: 耳蜗支持细胞基因治疗和再生的方法. Applicant: 苏州星奥拓维生物技术有限公司. The sequence listing filed with the application follows.

SEQUENCE LISTING (9 sequences)

SEQ ID NO: 1 - DNA, 1954 bp, synthetic construct
  source 1..1954: mol_type = other DNA
agggcacatgaggatgcagaccccagaccctggcacgtgccccgctcaggcacggccccacagctgcctcaggagggctggagagtggtggggggacctggtgccaggcagcagaggctggggtggggggctggctggccccttgcgctgccccccggcaccccggcctggctccatctctcccggccgcccagctgccggcacatccgcccaggcccagacatcaatccacaccaggcccttgctctgctctttcttttctgccctcctcttccctccccagcttgtatctttttttttttccttctctctctctctctattccaacatgtcattacagtagaaacaaaaagcgcggggacaatgcgggcattgacggcggccccctcccgccccctccccccgcggtgcgtgccagcactctttccacccgcccagggctggaaccgctgccaaaggagccctgctcataaacaagaggaaccagataaaccaggaacacaatagagggatttgttgcacttagaatggtgggaacaatgtcaacgtcgcgcgcagctgcttctaagcccccaccccaccaagtcctgccaagcagccccctcgcccctaagcccctctgatttatgaaaggtcagagggcatcatggctaaagggccccttcctcacatccctcgttaacccttcggacacaatggtcccttctctgggaggtggcggatgggggcgtgtgtcaagcgcagcacttcctggagcatcccagggacggctggtggaggtacagagggaggagcaggctcccaaatgcctttgggccggggctttgtccagagtaatgcctcattggaggaggccttctgaaatgacccccaagggtgtggtcagagcccactttgggtctacatgatgatgaccccaggctttctcgagcaagatggcggccgccagtgcaggcgctgggagagggagggcgccgcggccgccacggtcagcgcgcagccccggggtgcgggcgccggcggggggaggagggagtttgggtgggtggggggccgggaagagccagcgagaggggcagggaggggaacaaaaggtccctttgtggcgctgcgggagaagagggagcgcattacccaatgcccagaagccatgttggtaacaagagaaccattctctgcctcacttggaaaacaacttggagcagagagagacagggagagatttaaccccatgggcgcgggcgcaaggggctcaaggccacggcggaaggtggggaggagcgagggcacactcaacgcctggacgaccaatctctcaacccgtcccatcctgtgcccgggtggctcctgggtccagagcccatcggtacccaggaacatccaaactgagcagcccacaagacatgcgctcctccctcccgcccacctttatcttaggaaagatttttttttttttaactcgaatccttcaggtgaaaataaagcaacagcagcaacagaaaaaaaaaacgtagtcttcttcagggttaatatcagaagacaagcttgtgcggctttggccaatcagatgcgcccctggcagctataatatagtgctaaaggcagcctctctcacaagctctccaggcttgctaccatttaaaatcagactctttttgtcttttgattgctgtctcgcgacccaactccgatgtgttccgttatcagcggccggcagcctgccattccagcccctgtctgggtggggagcggtggagagtcccccgcagccgcggcgggcaaggttatataggaagagaaagagcgaggcagccagcgagggagagagcgagcgggcgagccggagcgaggaagggaaagcgcaagagagagcgcacacgcacacacccgccgcgcgcactcgcgcacggacccgcacggggacagctcggaagtcatcagttccatgggcgag

SEQ ID NO: 2 - DNA, 1365 bp, synthetic construct
  source 1..1365: mol_type = other DNA
agggcacatgaggatgcagaccccagaccctggcacgtgccccgctcaggcacggccccacagctgcctcaggagggctggagagtggtggggggacctggtgccaggcagcagaggctggggtggggggctggctggccccttgcgctgccccccggcaccccggcctggctccatctctcccggccgcccagctgccggcacatccgcccaggcccagacatcaatccacaccaggcccttgctctgctctttcttttctgccctcctcttccctccccagcttgtatctttttttttttccttctctctctctctctattccaacatgtcattacagtagaaacaaaaagcgcggggacaatgcgggcattgacggcggccccctcccgccccctccccccgcggtgcgtgccagcactctttccacccgcccagggctggaaccgctgccaaaggagccctgctcataaacaagaggaaccagataaaccaggaacacaatagagggatttgttgcacttagaatggtgggaacaatgtcaacgtcgcgcgcagctgcttctaagcccccaccccaccaagtcctgccaagcagccccctcgcccctaagcccctctgatttatgaaaggtcagagggcatcatggctaaagggccccttcctcacatccctcgttaacccttcggacacaatggtcccttctctgggaggtggcggatgggggcgtgtgtcaagcgcagcacttcctggagcatcccagggacggctggtggaggtacagagggaggagcaggctcccaaatgcctttgggccggggctttgtccagagtaatgcctcattggaggaggccttctgaaatgacccccaagggtgtggtcagagcccactttgggtctacatgatgatgaccccaggctttctcgagcaagatggcggccgccagtgcaggcgctgggagagggagggcgccgcggccgccacggtcagcgcgcagccccggggtgcgggcgccggcggggggaggagggagtttgggtgggtggggggccgggaagagccagcgagaggggcagggaggggaacaaaaggtccctttgtggcgctgcgggagaagagggagcgcattacccaatgcccagaagccatgttggtaacaagagaaccattctctgcctcacttggaaaacaacttggagcagagagagacagggagagatttaaccccatgggcgcgggcgcaaggggctcaaggccacggcggaaggtggggaggagcgagggcacactcaacgcctggacgaccaatctctcaacccgtcccatcctgtgcccgggtggctcctgggtccagagcccatc

SEQ ID NO: 3 - DNA, 589 bp, synthetic construct
  source 1..589: mol_type = other DNA
ggtacccaggaacatccaaactgagcagcccacaagacatgcgctcctccctcccgcccacctttatcttaggaaagatttttttttttttaactcgaatccttcaggtgaaaataaagcaacagcagcaacagaaaaaaaaaacgtagtcttcttcagggttaatatcagaagacaagcttgtgcggctttggccaatcagatgcgcccctggcagctataatatagtgctaaaggcagcctctctcacaagctctccaggcttgctaccatttaaaatcagactctttttgtcttttgattgctgtctcgcgacccaactccgatgtgttccgttatcagcggccggcagcctgccattccagcccctgtctgggtggggagcggtggagagtcccccgcagccgcggcgggcaaggttatataggaagagaaagagcgaggcagccagcgagggagagagcgagcgggcgagccggagcgaggaagggaaagcgcaagagagagcgcacacgcacacacccgccgcgcgcactcgcgcacggacccgcacggggacagctcggaagtcatcagttccatgggcgag

SEQ ID NO: 4 - DNA, 708 bp, synthetic construct
  source 1..708: mol_type = other DNA
atggtgtctaagggcgaggaggataacatggccagcctgcctgctacacacgagctgcacatcttcggaagcatcaacggcgtggactttgatatggtgggccagggaaccggcaacccaaacgacggatacgaggagctgaacctgaagagcacaaagggcgatctgcagttctccccctggattctggtgcctcacatcggatacggctttcaccagtacctgccatacccagacggaatgagcccattccaggctgctatggtggatggcagcggctaccaggtgcacaggaccatgcagtttgaggacggcgcctctctgaccgtgaactacagatacacatacgagggaagccacatcaagggcgaggcccaggtgaagggaaccggcttccctgctgacggaccagtgatgaccaactccctgacagccgctgactggtgccggtctaagaaaacataccctaacgataagaccatcatctctacattcaagtggagctacaccacaggaaacggcaagaggtacagatccaccgcccggaccacatacacatttgctaagccaatggccgctaactacctgaagaaccagcccatgtacgtgttccgcaagaccgagctgaagcactccaagacagagctgaacttcaaggagtggcagaaggcctttaccgacgtgatgggaatggatgagctgtacaag

SEQ ID NO: 5 - protein, 236 aa, synthetic construct
MVSKGEEDNMASLPATHELHIFGSINGVDFDMVGQGTGNPNDGYEELNLKSTKGDLQFSPWILVPHIGYGFHQYLPYPDGMSPFQAAMVDGSGYQVHRTMQFEDGASLTVNYRYTYEGSHIKGEAQVKGTGFPADGPVMTNSLTAADWCRSKKTYPNDKTIISTFKWSYTTGNGKRYRSTARTTYTFAKPMAANYLKNQPMYVFRKTELKHSKTELNFKEWQKAFTDVMGMDELYK

SEQ ID NO: 6 - DNA, 5416 bp, synthetic construct
  source 1..5416: mol_type = other DNA
cctgcaggcagctgcgcgctcgctcgctcactgaggccgcccgggcaaagcccgggcgtcgggcgacctttggtcgcccggcctcagtgagcgagcgagcgcgcagagagggagtggccaactccatcactaggggttcctgcggccgcacgcgtaagctttgcaaagatggataaagttttaaacagagaggaatctctcgagccattgacgtcaataatgacgtatgttcccatagtaacgccaatagggactttccattgacgtcaatgggtggagtatttacggtaaactgcccacttggcagtacatcaagtgtatcatatgccaagtacgccccctattgacgtcaatgacggtaaatggcccgcctggcattatgcccagtacatgaccttatgggactttcctacttggcagtacatctacgtattagtcatcgctattaccatggtcgaggtgagccccacgttctgcttcactctccccatctcccccccctccccacccccaattttgtatttatttattttttaattattttgtgcagcgatgggggcgggggggggggggggggggcggggcgaggcggagaggtgcggcggcagccaatcagagcggcgcgctccgaaagtttccttttatggcgaggcggcggcggcggcggccctataaaaagcgaagcgcgcggcgggcgggagtcgctgcgcgctgccttcgccccgtgccccgctccgccgccgcctcgcgccgcccgccccggctctgactgaccgcgttactcccacaggtgagcgggcgggacggcccttctcctccgggctgtaattagcgcttggtttaatgacggcttgtttcttttctgtggctgcgtgaaagccttgaggggctccgggagggccctttgtgcggggggagcggctcggggctgtccgcggggggacggctgccttcgggggggacggggcagggcggggttcggcttctggcgtgtgaccggcggctctagagcctctgctaaccatgttcatgccttcttctttttcctacagctcctgggcaacgtgctggttattgtgctgtctcatcattttggcaaagaattggatcgaattcgccaccatgccaaagaagaagcgtaaggtaggatctggagtgagcaagggcgaggagctgttcaccggggtggtgcccatcctggtcgagctggacggcgacgtaaacggccacaagttcagcgtgtccggcgagggcgagggcgatgccacctacggcaagctgaccctgaagttcatctgcaccaccggcaagctgcccgtgccctggcccaccctcgtgaccaccctgacctacggcgtgcagtgcttcagccgctaccccgaccacatgaagcagcacgacttcttcaagtccgccatgcccgaaggctacgtccaggagcgcaccatcttcttcaaggacgacggcaactacaagacccgcgccgaggtgaagttcgagggcgacaccctggtgaaccgcatcgagctgaagggcatcgacttcaaggaggacggcaacatcctggggcacaagctggagtacaactacaacagccacaacgtctatatcatggccgacaagcagaagaacggcatcaaggtgaacttcaagatccgccacaacatcgaggacggcagcgtgcagctcgccgaccactaccagcagaacacccccatcggcgacggccccgtgctgctgcccgacaaccactacctgagcacccagtccgccctgagcaaagaccccaacgagaagcgcgatcacatggtcctgctggagttcgtgaccgccgccgggatcactctcggcatggacgagctgtacaagggatccggatacccatacgatgttcctgactatgcgtgatatcaagcttatcgataatcaacctctggattacaaaatttgtgaaagattgactggtattcttaactatgttgctccttttacgctatgtggatacgctgctttaatgcctttgtatcatgctattgcttcccgtatggctttcattttctcctccttgtataaatcctggttgctgtctctttatgaggagttgtggcccgttgtcaggcaacgtggcgtggtgtgcactgtgtttgctgacgcaacccccactggttggggcattgccaccacctgtcagctcctttccgggactttcgctttccccctccctattgccacggcggaactcatcgccgcctgccttgcccgctgctggacaggggctcggctgttgggcactgacaattccgtggtgttgtcggggaaatcatcgtcctttccttggctgctcgcctgtgttgccacctggattctgcgcgggacgtccttctgctacgtcccttcggccctcaatccagcggaccttccttcccgcggcctgctgccggctctgcggcctcttccgcgacttcgccttcgccctcagacgagtcggatctccctttgggccgcctccccgcagatctaacttgtttattgcagcttataatggttacaaataaagcaatagcatcacaaatttcacaaataaagcatttttttcactgcattctagttgtggtttgtccaaactcatcaatgtatcttatcatgtctggctagacacgtgcggaccgagcggccgcaggaacccctagtgatggagttggccactccctctctgcgcgctcgctcgctcactgaggccgggcgaccaaaggtcgcccgacgcccgggctttgcccgggcggcctcagtgagcgagcgagcgcgcagctgcctgcaggggcgcctgatgcggtattttctccttacgcatctgtgcggtatttcacaccgcatacgtcaaagcaaccatagtacgcgccctgtagcggcgcattaagcgcggcgggtgtggtggttacgcgcagcgtgaccgctacacttgccagcgccctagcgcccgctcctttcgctttcttcccttcctttctcgccacgttcgccggctttccccgtcaagctctaaatcgggggctccctttagggttccgatttagtgctttacggcacctcgaccccaaaaaacttgatttgggtgatggttcacgtagtgggccatcgccctgatagacggtttttcgccctttgacgttggagtccacgttctttaatagtggactcttgttccaaactggaacaacactcaaccctatctcgggctattcttttgatttataagggattttgccgatttcggcctattggttaaaaaatgagctgatttaacaaaaatttaacgcgaattttaacaaaatattaacgtttacaattttatggtgcactctcagtacaatctgctctgatgccgcatagttaagccagccccgacacccgccaacacccgctgacgcgccctgacgggcttgtctgctcccggcatccgcttacagacaagctgtgaccgtctccgggagctgcatgtgtcagaggttttcaccgtcatcaccgaaacgcgcgagacgaaagggcctcgtgatacgcctatttttataggttaatgtcatgataataatggtttcttagacgtcaggtggcacttttcggggaaatgtgcgcggaacccctatttgtttatttttctaaatacattcaaatatgtatccgctcatgagacaataaccctgataaatgcttcaataatattgaaaaaggaagagtatgagtattcaacatttccgtgtcgcccttattcccttttttgcggcattttgccttcctgtttttgctcacccagaaacgctggtgaaagtaaaagatgctgaagatcagttgggtgcacgagtgggttacatcgaactggatctcaacagcggtaagatccttgagagttttcgccccgaagaacgttttccaatgatgagcacttttaaagttctgctatgtggcgcggtattatcccgtattgacgccgggcaagagcaactcggtcgccgcatacactattctcagaatgacttggttgagtactcaccagtcacagaaaagcatcttacggatggcatgacagtaagagaattatgcagtgctgccataaccatgagtgataacactgcggccaacttacttctgacaacgatcggaggaccgaaggagctaaccgcttttttgcacaacatgggggatcatgtaactcgccttgatcgttgggaaccggagctgaatgaagccataccaaacgacgagcgtgacaccacgatgcctgtagcaatggcaacaacgttgcgcaaactattaactggcgaactacttactctagcttcccggcaacaattaatagactggatggaggcggataaagttgcaggaccacttctgcgctcggcccttccggctggctggtttattgctgataaatctggagccggtgagcgtgggtctcgcggtatcattgcagcactggggccagatggtaagccctcccgtatcgtagttatctacacgacggggagtcaggcaactatggatgaacgaaatagacagatcgctgagataggtgcctcactgattaagcattggtaactgtcagaccaagtttactcatatatactttagattgatttaaaacttcatttttaatttaaaaggatctaggtgaagatcctttttgataatctcatgaccaaaatcccttaacgtgagttttcgttccactgagcgtcagaccccgtagaaaagatcaaaggatcttcttgagatcctttttttctgcgcgtaatctgctgcttgcaaacaaaaaaaccaccgctaccagcggtggtttgtttgccggatcaagagctaccaactctttttccgaaggtaactggcttcagcagagcgcagataccaaatactgtccttctagtgtagccgtagttaggccaccacttcaagaactctgtagcaccgcctacatacctcgctctgctaatcctgttaccagtggctgctgccagtggcgataagtcgtgtcttaccgggttggactcaagacgatagttaccggataaggcgcagcggtcgggctgaacggggggttcgtgcacacagcccagcttggagcgaacgacctacaccgaactgagatacctacagcgtgagctatgagaaagcgccacgcttcccgaagggagaaaggcggacaggtatccggtaagcggcagggtcggaacaggagagcgcacgagggagcttccagggggaaacgcctggtatctttatagtcctgtcgggtttcgccacctctgacttgagcgtcgatttttgtgatgctcgtcaggggggcggagcctatggaaaaacgccagcaacgcggcctttttacggttcctggccttttgctggccttttgctcacatgt

SEQ ID NO: 7 - DNA, 6130 bp, synthetic construct
  source 1..6130: mol_type = other DNA
cctgcaggcagctgcgcgctcgctcgctcactgaggccgcccgggcaaagcccgggcgtcgggcgacctttggtcgcccggcctcagtgagcgagcgagcgcgcagagagggagtggccaactccatcactaggggttcctgcggccgcacgcgtaagctttgcaaagatggataaagttttaaacagagaggaatctctcgagccattgacgtcaataatgacgtatgttcccatagtaacgccaatagggactttccattgacgtcaatgggtggagtatttacggtaaactgcccacttggcagtacatcaagtgtatcatatgccaagtacgccccctattgacgtcaatgacggtaaatggcccgcctggcattatgcccagtacatgaccttatgggactttcctacttggcagtacatctacgtattagtcatcgctattaccatggtcgaggtgagccccacgttctgcttcactctccccatctcccccccctccccacccccaattttgtatttatttattttttaattattttgtgcagcgatgggggcgggggggggggggggggggcggggcgaggcggagaggtgcggcggcagccaatcagagcggcgcgctccgaaagtttccttttatggcgaggcggcggcggcggcggccctataaaaagcgaagcgcgcggcgggcgggagtcgctgcgcgctgccttcgccccgtgccccgctccgccgccgcctcgcgccgcccgccccggctctgactgaccgcgttactcccacaggtgagcgggcgggacggcccttctcctccgggctgtaattagcgcttggtttaatgacggcttgtttcttttctgtggctgcgtgaaagccttgaggggctccgggagggccctttgtgcggggggagcggctcggggctgtccgcggggggacggctgccttcgggggggacggggcagggcggggttcggcttctggcgtgtgaccggcggctctagagcctctgctaaccatgttcatgccttcttctttttcctacagctcctgggcaacgtgctggttattgtgctgtctcatcattttggcaaagaattggatcgaattcgccaccatgccaaagaagaagcgtaaggtaggatctggagtgagcaagggcgaggagctgttcaccggggtggtgcccatcctggtcgagctggacggcgacgtaaacggccacaagttcagcgtgtccggcgagggcgagggcgatgccacctacggcaagctgaccctgaagttcatctgcaccaccggcaagctgcccgtgccctggcccaccctcgtgaccaccctgacctacggcgtgcagtgcttcagccgctaccccgaccacatgaagcagcacgacttcttcaagtccgccatgcccgaaggctacgtccaggagcgcaccatcttcttcaaggacgacggcaactacaagacccgcgccgaggtgaagttcgagggcgacaccctggtgaaccgcatcgagctgaagggcatcgacttcaaggaggacggcaacatcctggggcacaagctggagtacaactacaacagccacaacgtctatatcatggccgacaagcagaagaacggcatcaaggtgaacttcaagatccgccacaacatcgaggacggcagcgtgcagctcgccgaccactaccagcagaacacccccatcggcgacggccccgtgctgctgcccgacaaccactacctgagcacccagtccgccctgagcaaagaccccaacgagaagcgcgatcacatggtcctgctggagttcgtgaccgccgccgggatcactctcggcatggacgagctgtacaagggttccggagccaccaacttttctctgctgaagcaggctggcgacgtggaggagaacccaggacctggatccatggattggggcacactccagagcatcctcgggggtgtcaacaaacactccaccagcattggaaagatctggctcacggtcctcttcatcttccgcatcatgatcctcgtggtggctgcaaaggaggtgtggggagatgagcaagccgattttgtctgcaacacgctccagcctggctgcaagaatgtatgctacgaccaccacttccccatctctcacatccggctctgggctctgcagctgatcatggtgtccacgccagccctcctggtagctatgcatgtggcctaccggagacatgaaaagaaacggaagttcatgaagggagagataaagaacgagtttaaggacatcgaagagatcaaaacccagaaggtccgtatcgaagggtccctgtggtggacctacaccaccagcatcttcttccgggtcatctttgaagccgtcttcatgtacgtcttttacatcatgtacaatggcttcttcatgcaacgtctggtgaaatgcaacgcttggccctgccccaatacagtggactgcttcatttccaggcccacagaaaagactgtcttcaccgtgtttatgatttctgtgtctggaatttgcattctgctaaatatcacagagctgtgctatttgttcgttaggtattgctcaggaaagtccaaaagaccagtctgatatcaagcttatcgataatcaacctctggattacaaaatttgtgaaagattgactggtattcttaactatgttgctccttttacgctatgtggatacgctgctttaatgcctttgtatcatgctattgcttcccgtatggctttcattttctcctccttgtataaatcctggttgctgtctctttatgaggagttgtggcccgttgtcaggcaacgtggcgtggtgtgcactgtgtttgctgacgcaacccccactggttggggcattgccaccacctgtcagctcctttccgggactttcgctttccccctccctattgccacggcggaactcatcgccgcctgccttgcccgctgctggacaggggctcggctgttgggcactgacaattccgtggtgttgtcggggaaatcatcgtcctttccttggctgctcgcctgtgttgccacctggattctgcgcgggacgtccttctgctacgtcccttcggccctcaatccagcggaccttccttcccgcggcctgctgccggctctgcggcctcttccgcgacttcgccttcgccctcagacgagtcggatctccctttgggccgcctccccgcagatctaacttgtttattgcagcttataatggttacaaataaagcaatagcatcacaaatttcacaaataaagcatttttttcactgcattctagttgtggtttgtccaaactcatcaatgtatcttatcatgtctggctagacacgtgcggaccgagcggccgcaggaacccctagtgatggagttggccactccctctctgcgcgctcgctcgctcactgaggccgggcgaccaaaggtcgcccgacgcccgggctttgcccgggcggcctcagtgagcgagcgagcgcgcagctgcctgcaggggcgcctgatgcggtattttctccttacgcatctgtgcggtatttcacaccgcatacgtcaaagcaaccatagtacgcgccctgtagcggcgcattaagcgcggcgggtgtggtggttacgcgcagcgtgaccgctacacttgccagcgccctagcgcccgctcctttcgctttcttcccttcctttctcgccacgttcgccggctttccccgtcaagctctaaatcgggggctccctttagggttccgatttagtgctttacggcacctcgaccccaaaaaacttgatttgggtgatggttcacgtagtgggccatcgccctgatagacggtttttcgccctttgacgttggagtccacgttctttaatagtggactcttgttccaaactggaacaacactcaaccctatctcgggctattcttttgatttataagggattttgccgatttcggcctattggttaaaaaatgagctgatttaacaaaaatttaacgcgaattttaacaaaatattaacgtttacaattttatggtgcactctcagtacaatctgctctgatgccgcatagttaagccagccccgacacccgccaacacccgctgacgcgccctgacgggcttgtctgctcccggcatccgcttacagacaagctgtgaccgtctccgggagctgcatgtgtcagaggttttcaccgtcatcaccgaaacgcgcgagacgaaagggcctcgtgatacgcctatttttataggttaatgtcatgataataatggtttcttagacgtcaggtggcacttttcggggaaatgtgcgcggaacccctatttgtttatttttctaaatacattcaaatatgtatccgctcatgagacaataaccctgataaatgcttcaataatattgaaaaaggaagagtatgagtattcaacatttccgtgtcgcccttattcccttttttgcggcattttgccttcctgtttttgctcacccagaaacgctggtgaaagtaaaagatgctgaagatcagttgggtgcacgagtgggttacatcgaactggatctcaacagcggtaagatccttgagagttttcgccccgaagaacgttttccaatgatgagcacttttaaagttctgctatgtggcgcggtattatcccgtattgacgccgggcaagagcaactcggtcgccgcatacactattctcagaatgacttggttgagtactcaccagtcacagaaaagcatcttacggatggcatgacagtaagagaattatgcagtgctgccataaccatgagtgataacactgcggccaacttacttctgacaacgatcggaggaccgaaggagctaaccgcttttttgcacaacatgggggatcatgtaactcgccttgatcgttgggaaccggagctgaatgaagccataccaaacgacgagcgtgacaccacgatgcctgtagcaatggcaacaacgttgcgcaaactattaactggcgaactacttactctagcttcccggcaacaattaatagactggatggaggcggataaagttgcaggaccacttctgcgctcggcccttccggctggctggtttattgctgataaatctggagccggtgagcgtgggtctcgcggtatcattgcagcactggggccagatggtaagccctcccgtatcgtagttatctacacgacggggagtcaggcaactatggatgaacgaaatagacagatcgctgagataggtgcctcactgattaagcattggtaactgtcagaccaagtttactcatatatactttagattgatttaaaacttcatttttaatttaaaaggatctaggtgaagatcctttttgataatctcatgaccaaaatcccttaacgtgagttttcgttccactgagcgtcagaccccgtagaaaagatcaaaggatcttcttgagatcctttttttctgcgcgtaatctgctgcttgcaaacaaaaaaaccaccgctaccagcggtggtttgtttgccggatcaagagctaccaactctttttccgaaggtaactggcttcagcagagcgcagataccaaatactgtccttctagtgtagccgtagttaggccaccacttcaagaactctgtagcaccgcctacatacctcgctctgctaatcctgttaccagtggctgctgccagtggcgataagtcgtgtcttaccgggttggactcaagacgatagttaccggataaggcgcagcggtcgggctgaacggggggttcgtgcacacagcccagcttggagcgaacgacctacaccgaactgagatacctacagcgtgagctatgagaaagcgccacgcttcccgaagggagaaaggcggacaggtatccggtaagcggcagggtcggaacaggagagcgcacgagggagcttccagggggaaacgcctggtatctttatagtcctgtcgggtttcgccacctctgacttgagcgtcgatttttgtgatgctcgtcaggggggcggagcctatggaaaaacgccagcaacgcggcctttttacggttcctggccttttgctggccttttgctcacatgt

SEQ ID NO: 8 - DNA, 6430 bp, synthetic construct
  source 1..6430: mol_type = other DNA
cctgcaggcagctgcgcgctcgctcgctcactgaggccgcccgggcaaagcccgggcgtcgggcgacctttggtcgcccggcctcagtgagcgagcgagcgcgcagagagggagtggccaactccatcactaggggttcctgcggccgcacgcgttctcgattctagatttacggtacagggcacatgaggatgcagaccccagaccctggcacgtgccccgctcaggcacggccccacagctgcctcaggagggctggagagtggtggggggacctggtgccaggcagcagaggctggggtggggggctggctggccccttgcgctgccccccggcaccccggcctggctccatctctcccggccgcccagctgccggcacatccgcccaggcccagacatcaatccacaccaggcccttgctctgctctttcttttctgccctcctcttccctccccagcttgtatctttttttttttccttctctctctctctctattccaacatgtcattacagtagaaacaaaaagcgcggggacaatgcgggcattgacggcggccccctcccgccccctccccccgcggtgcgtgccagcactctttccacccgcccagggctggaaccgctgccaaaggagccctgctcataaacaagaggaaccagataaaccaggaacacaatagagggatttgttgcacttagaatggtgggaacaatgtcaacgtcgcgcgcagctgcttctaagcccccaccccaccaagtcctgccaagcagccccctcgcccctaagcccctctgatttatgaaaggtcagagggcatcatggctaaagggccccttcctcacatccctcgttaacccttcggacacaatggtcccttctctgggaggtggcggatgggggcgtgtgtcaagcgcagcacttcctggagcatcccagggacggctggtggaggtacagagggaggagcaggctcccaaatgcctttgggccggggctttgtccagagtaatgcctcattggaggaggccttctgaaatgacccccaagggtgtggtcagagcccactttgggtctacatgatgatgaccccaggctttctcgagcaagatggcggccgccagtgcaggcgctgggagagggagggcgccgcggccgccacggtcagcgcgcagccccggggtgcgggcgccggcggggggaggagggagtttgggtgggtggggggccgggaagagccagcgagaggggcagggaggggaacaaaaggtccctttgtggcgctgcgggagaagagggagcgcattacccaatgcccagaagccatgttggtaacaagagaaccattctctgcctcacttggaaaacaacttggagcagagagagacagggagagatttaaccccatgggcgcgggcgcaaggggctcaaggccacggcggaaggtggggaggagcgagggcacactcaacgcctggacgaccaatctctcaacccgtcccatcctgtgcccgggtggctcctgggtccagagcccatcggtacccaggaacatccaaactgagcagcccacaagacatgcgctcctccctcccgcccacctttatcttaggaaagatttttttttttttaactcgaatccttcaggtgaaaataaagcaacagcagcaacagaaaaaaaaaacgtagtcttcttcagggttaatatcagaagacaagcttgtgcggctttggccaatcagatgcgcccctggcagctataatatagtgctaaaggcagcctctctcacaagctctccaggcttgctaccatttaaaatcagactctttttgtcttttgattgctgtctcgcgacccaactccgatgtgttccgttatcagcggccggcagcctgccattccagcccctgtctgggtggggagcggtggagagtcccccgcagccgcggcgggcaaggttatataggaagagaaagagcgaggcagccagcgagggagagagcgagcgggcgagccggagcgaggaagggaaagcgcaagagagagcgcacacgcacacacccgccgcgcgcactcgcgcacggacccgcacggggacagctcggaagtcatcagttccatgggcgagctagcgaattcgccaccatgaagcggacagctgatggcagcgagttcgagtcccccaagaagaagaggaaggtggagatggtgtctaagggcgaggaggataacatggccagcctgcctgctacacacgagctgcacatcttcggaagcatcaacggcgtggactttgatatggtgggccagggaaccggcaacccaaacgacggatacgaggagctgaacctgaagagcacaaagggcgatctgcagttctccccctggattctggtgcctcacatcggatacggctttcaccagtacctgccatacccagacggaatgagcccattccaggctgctatggtggatggcagcggctaccaggtgcacaggaccatgcagtttgaggacggcgcctctctgaccgtgaactacagatacacatacgagggaagccacatcaagggcgaggcccaggtgaagggaaccggcttccctgctgacggaccagtgatgaccaactccctgacagccgctgactggtgccggtctaagaaaacataccctaacgataagaccatcatctctacattcaagtggagctacaccacaggaaacggcaagaggtacagatccaccgcccggaccacatacacatttgctaagccaatggccgctaactacctgaagaaccagcccatgtacgtgttccgcaagaccgagctgaagcactccaagacagagctgaacttcaaggagtggcagaaggcctttaccgacgtgatgggaatggatgagctgtacaagtgagatatcaagcttatcgataatcaacctctggattacaaaatttgtgaaagattgactggtattcttaactatgttgctccttttacgctatgtggatacgctgctttaatgcctttgtatcatgctattgcttcccgtatggctttcattttctcctccttgtataaatcctggttgctgtctctttatgaggagttgtggcccgttgtcaggcaacgtggcgtggtgtgcactgtgtttgctgacgcaacccccactggttggggcattgccaccacctgtcagctcctttccgggactttcgctttccccctccctattgccacggcggaactcatcgccgcctgccttgcccgctgctggacaggggctcggctgttgggcactgacaattccgtggtgttgtcggggaaatcatcgtcctttccttggctgctcgcctgtgttgccacctggattctgcgcgggacgtccttctgctacgtcccttcggccctcaatccagcggaccttccttcccgcggcctgctgccggctctgcggcctcttccgcgacttcgccttcgccctcagacgagtcggatctccctttgggccgcctccccgcagatctaacttgtttattgcagcttataatggttacaaataaagcaatagcatcacaaatttcacaaataaagcatttttttcactgcattctagttgtggtttgtccaaactcatcaatgtatcttatcatgtctggctagacacgtgcggaccgagcggccgcaggaacccctagtgatggagttggccactccctctctgcgcgctcgctcgctcactgaggccgggcgaccaaaggtcgcccgacgcccgggctttgcccgggcggcctcagtgagcgagcgagcgcgcagctgcctgcaggggcgcctgatgcggtattttctccttacgcatctgtgcggtatttcacaccgcatacgtcaaagcaaccatagtacgcgccctgtagcggcgcattaagcgcggcgggtgtggtggttacgcgcagcgtgaccgctacacttgccagcgccctagcgcccgctcctttcgctttcttcccttcctttctcgccacgttcgccggctttccccgtcaagctctaaatcgggggctccctttagggttccgatttagtgctttacggcacctcgaccccaaaaaacttgatttgggtgatggttcacgtagtgggccatcgccctgatagacggtttttcgccctttgacgttggagtccacgttctttaatagtggactcttgttccaaactggaacaacactcaaccctatctcgggctattcttttgatttataagggattttgccgatttcggcctattggttaaaaaatgagctgatttaacaaaaatttaacgcgaattttaacaaaatattaacgtttacaattttatggtgcactctcagtacaatctgctctgatgccgcatagttaagccagccccgacacccgccaacacccgctgacgcgccctgacgggcttgtctgctcccggcatccgcttacagacaagctgtgaccgtctccgggagctgcatgtgtcagaggttttcaccgtcatcaccgaaacgcgcgagacgaaagggcctcgtgatacgcctatttttataggttaatgtcatgataataatggtttcttagacgtcaggtggcacttttcggggaaatgtgcgcggaacccctatttgtttatttttctaaatacattcaaatatgtatccgctcatgagacaataaccctgataaatgcttcaataatattgaaaaaggaagagtatgagtattcaacatttccgtgtcgcccttattcccttttttgcggcattttgccttcctgtttttgctcacccagaaacgctggtgaaagtaaaagatgctgaagatcagttgggtgcacgagtgggttacatcgaactggatctcaacagcggtaagatccttgagagttttcgccccgaagaacgttttccaatgatgagcacttttaaagttctgctatgtggcgcggtattatcccgtattgacgccgggcaagagcaactcggtcgccgcatacactattctcagaatgacttggttgagtactcaccagtcacagaaaagcatcttacggatggcatgacagtaagagaattatgcagtgctgccataaccatgagtgataacactgcggccaacttacttctgacaacgatcggaggaccgaaggagctaaccgcttttttgcacaacatgggggatcatgtaactcgccttgatcgttgggaaccggagctgaatgaagccataccaaacgacgagcgtgacaccacgatgcctgtagcaatggcaacaacgttgcgcaaactattaactggcgaactacttactctagcttcccggcaacaattaatagactggatggaggcggataaagttgcaggaccacttctgcgctcggcccttccggctggctggtttattgctgataaatctggagccggtgagcgtgggtctcgcggtatcattgcagcactggggccagatggtaagccctcccgtatcgtagttatctacacgacggggagtcaggcaactatggatgaacgaaatagacagatcgctgagataggtgcctcactgattaagcattggtaactgtcagaccaagtttactcatatatactttagattgatttaaaacttcatttttaatttaaaaggatctaggtgaagatcctttttgataatctcatgaccaaaatcccttaacgtgagttttcgttccactgagcgtcagaccccgtagaaaagatcaaaggatcttcttgagatcctttttttctgcgcgtaatctgctgcttgcaaacaaaaaaaccaccgctaccagcggtggtttgtttgccggatcaagagctaccaactctttttccgaaggtaactggcttcagcagagcgcagataccaaatactgtccttctagtgtagccgtagttaggccaccacttcaagaactctgtagcaccgcctacatacctcgctctgctaatcctgttaccagtggctgctgccagtggcgataagtcgtgtcttaccgggttggactcaagacgatagttaccggataaggcgcagcggtcgggctgaacggggggttcgtgcacacagcccagcttggagcgaacgacctacaccgaactgagatacctacagcgtgagctatgagaaagcgccacgcttcccgaagggagaaaggcggacaggtatccggtaagcggcagggtcggaacaggagagcgcacgagggagcttccagggggaaacgcctggtatctttatagtcctgtcgggtttcgccacctctgacttgagcgtcgatttttgtgatgctcgtcaggggggcggagcctatggaaaaacgccagcaacgcggcctttttacggttcctggccttttgctggccttttgctcacatgt

SEQ ID NO: 9 - DNA, 6340 bp, synthetic construct
  source 1..6340: mol_type = other DNA
cctgcaggcagctgcgcgctcgctcgctcactgaggccgcccgggcaaagcccgggcgtcgggcgacctttggtcgcccggcctcagtgagcgagcgagcgcgcagagagggagtggccaactccatcactaggggttcctgcggccgcacgcgttctcgattctagatttacggtacagggcacatgaggatgcagaccccagaccctggcacgtgccccgctcaggcacggccccacagctgcctcaggagggctggagagtggtggggggacctggtgccaggcagcagaggctggggtggggggctggctggccccttgcgctgccccccggcaccccggcctggctccatctctcccggccgcccagctgccggcacatccgcccaggcccagacatcaatccacaccaggcccttgctctgctctttcttttctgccctcctcttccctccccagcttgtatctttttttttttccttctctctctctctctattccaacatgtcattacagtagaaacaaaaagcgcggggacaatgcgggcattgacggcggccccctcccgccccctccccccgcggtgcgtgccagcactctttccacccgcccagggctggaaccgctgccaaaggagccctgctcataaacaagaggaaccagataaaccaggaacacaatagagggatttgttgcacttagaatggtgggaacaatgtcaacgtcgcgcgcagctgcttctaagcccccaccccaccaagtcctgccaagcagccccctcgcccctaagcccctctgatttatgaaaggtcagagggcatcatggctaaagggccccttcctcacatccctcgttaacccttcggacacaatggtcccttctctgggaggtggcggatgggggcgtgtgtcaagcgcagcacttcctggagcatcccagggacggctggtggaggtacagagggaggagcaggctcccaaatgcctttgggccggggctttgtccagagtaatgcctcattggaggaggccttctgaaatgacccccaagggtgtggtcagagcccactttgggtctacatgatgatgaccccaggctttctcgagcaagatggcggccgccagtgcaggcgctgggagagggagggcgccgcggccgccacggtcagcgcgcagccccggggtgcgggcgccggcggggggaggagggagtttgggtgggtggggggccgggaagagccagcgagaggggcagggaggggaacaaaaggtccctttgtggcgctgcgggagaagagggagcgcattacccaatgcccagaagccatgttggtaacaagagaaccattctctgcctcacttggaaaacaacttggagcagagagagacagggagagatttaaccccatgggcgcgggcgcaaggggctcaaggccacggcggaaggtggggaggagcgagggcacactcaacgcctggacgaccaatctctcaacccgtcccatcctgtgcccgggtggctcctgggtccagagcccatcggtacccaggaacatccaaactgagcagcccacaagacatgcgctcctccctcccgcccacctttatcttaggaaagatttttttttttttaactcgaatccttcaggtgaaaataaagcaacagcagcaacagaaaaaaaaaacgtagtcttcttcagggttaatatcagaagacaagcttgtgcggctttggccaatcagatgcgcccctggcagctataatatagtgctaaaggcagcctctctcacaagctctccaggcttgctaccatttaaaatcagactctttttgtcttttgattgctgtctcgcgacccaactccgatgtgttccgttatcagcggccggcagcctgccattccagcccctgtctgggtggggagcggtggagagtcccccgcagccgcggcgggcaaggttatataggaagagaaagagcgaggcagccagcgagggagagagcgagcgggcgagccggagcgaggaagggaaagcgcaagagagagcgcacacgcacacacccgccgcgcgcactcgcgcacggacccgcacggggacagctcggaagtcatcagttccatgggcgagctagcgaattcgccaccatggattggggcacgctgcagacgatcctggggggtgtgaacaaacactccaccagcattggaaagatctggctcaccgtcctcttcatttttcgcattatgatcctcgttgtggctgcaaaggaggtgtggggagatgagcaggccgactttgtctgcaacaccctgcagccaggctgcaagaacgtgtgctacgatcactacttccccatctcccacatccggctatgggccctgcagctgatcttcgtgtccacgccagcgctcctagtggccatgcacgtggcctaccggagacatgagaagaagaggaagttcatcaagggggagataaagagtgaatttaaggacatcgaggagatcaaaacccagaaggtccgcatcgaaggctccctgtggtggacctacacaagcagcatcttcttccgggtcatcttcgaagccgccttcatgtacgtcttctatgtcatgtacgacggcttctccatgcagcggctggtgaagtgcaacgcctggccttgtcccaacactgtggactgctttgtgtcccggcccacggagaaaaccgtatttacagtcttcatgattgcagtgtctggaatttgcatcctgctgaatgtcactgaattgtgttatttgctaattagatattgttctgggaagtcaaaaaagccagtttaagatatcaagcttatcgataatcaacctctggattacaaaatttgtgaaagattgactggtattcttaactatgttgctccttttacgctatgtggatacgctgctttaatgcctttgtatcatgctattgcttcccgtatggctttcattttctcctccttgtataaatcctggttgctgtctctttatgaggagttgtggcccgttgtcaggcaacgtggcgtggtgtgcactgtgtttgctgacgcaacccccactggttggggcattgccaccacctgtcagctcctttccgggactttcgctttccccctccctattgccacggcggaactcatcgccgcctgccttgcccgctgctggacaggggctcggctgttgggcactgacaattccgtggtgttgtcggggaaatcatcgtcctttccttggctgctcgcctgtgttgccacctggattctgcgcgggacgtccttctgctacgtcccttcggccctcaatccagcggaccttccttcccgcggcctgctgccggctctgcggcctcttccgcgacttcgccttcgccctcagacgagtcggatctccctttgggccgcctccccgcagatctaacttgtttattgcagcttataatggttacaaataaagcaatagcatcacaaatttcacaaataaagcatttttttcactgcattctagttgtggtttgtccaaactcatcaatgtatcttatcatgtctggctagacacgtgcggaccgagcggccgcaggaacccctagtgatggagttggccactccctctctgcgcgctcgctcgctcactgaggccgggcgaccaaaggtcgcccgacgcccgggctttgcccgggcggcctcagtgagcgagcgagcgcgcagctgcctgcaggggcgcctgatgcggtattttctccttacgcatctgtgcggtatttcacaccgcatacgtcaaagcaaccatagtacgcgccctgtagcggcgcattaagcgcggcgggtgtggtggttacgcgcagcgtgaccgctacacttgccagcgccctagcgcccgctcctttcgctttcttcccttcctttctcgccacgttcgccggctttccccgtcaagctctaaatcgggggctccctttagggttccgatttagtgctttacggcacctcgaccccaaaaaacttgatttgggtgatggttcacgtagtgggccatcgccctgatagacggtttttcgccctttgacgttggagtccacgttctttaatagtggactcttgttccaaactggaacaacactcaaccctatctcgggctattcttttgatttataagggattttgccgatttcggcctattggttaaaaaatgagctgatttaacaaaaatttaacgcgaattttaacaaaatattaacgtttacaattttatggtgcactctcagtacaatctgctctgatgccgcatagttaagccagccccgacacccgccaacacccgctgacgcgccctgacgggcttgtctgctcccggcatccgcttacagacaagctgtgaccgtctccgggagctgcatgtgtcagaggttttcaccgtcatcaccgaaacgcgcgagacgaaagggcctcgtgatacgcctatttttataggttaatgtcatgataataatggtttcttagacgtcaggtggcacttttcggggaaatgtgcgcggaacccctatttgtttatttttctaaatacattcaaatatgtatccgctcatgagacaataaccctgataaatgcttcaataatattgaaaaaggaagagtatgagtattcaacatttccgtgtcgcccttattcccttttttgcggcattttgccttcctgtttttgctcacccagaaacgctggtgaaagtaaaagatgctgaagatcagttgggtgcacgagtgggttacatcgaactggatctcaacagcggtaagatccttgagagttttcgccccgaagaacgttttccaatgatgagcacttttaaagttctgctatgtggcgcggtattatcccgtattgacgccgggcaagagcaactcggtcgccgcatacactattctcagaatgacttggttgagtactcaccagtcacagaaaagcatcttacggatggcatgacagtaagagaattatgcagtgctgccataaccatgagtgataacactgcggccaacttacttctgacaacgatcggaggaccgaaggagctaaccgcttttttgcacaacatgggggatcatgtaactcgccttgatcgttgggaaccggagctgaatgaagccataccaaacgacgagcgtgacaccacgatgcctgtagcaatggcaacaacgttgcgcaaactattaactggcgaactacttactctagcttcccggcaacaattaatagactggatggaggcggataaagttgcaggaccacttctgcgctcggcccttccggctggctggtttattgctgataaatctggagccggtgagcgtgggtctcgcggtatcattgcagcactggggccagatggtaagccctcccgtatcgtagttatctacacgacggggagtcaggcaactatggatgaacgaaatagacagatcgctgagataggtgcctcactgattaagcattggtaactgtcagaccaagtttactcatatatactttagattgatttaaaacttcatttttaatttaaaaggatctaggtgaagatcctttttgataatctcatgaccaaaatcccttaacgtgagttttcgttccactgagcgtcagaccccgtagaaaagatcaaaggatcttcttgagatcctttttttctgcgcgtaatctgctgcttgcaaacaaaaaaaccaccgctaccagcggtggtttgtttgccggatcaagagctaccaactctttttccgaaggtaactggcttcagcagagcgcagataccaaatactgtccttctagtgtagccgtagttaggccaccacttcaagaactctgtagcaccgcctacatacctcgctctgctaatcctgttaccagtggctgctgccagtggcgataagtcgtgtcttaccgggttggactcaagacgatagttaccggataaggcgcagcggtcgggctgaacggggggttcgtgcacacagcccagcttggagcgaacgacctacaccgaactgagatacctacagcgtgagctatgagaaagcgccacgcttcccgaagggagaaaggcggacaggtatccggtaagcggcagggtcggaacaggagagcgcacgagggagcttccagggggaaacgcctggtatctttatagtcctgtcgggtttcgccacctctgacttgagcgtcgatttttgtgatgctcgtcaggggggcggagcctatggaaaaacgccagcaacgcggcctttttacggttcctggccttttgctggccttttgctcacatgt